European Patent Application EP 4 450 648 A2, published October 23, 2024. Title: DETERMINING A PHYSIOLOGICAL CONDITION IN AN INDIVIDUAL BY ANALYZING CELL-FREE DNA FRAGMENT ENDPOINTS IN A BIOLOGICAL SAMPLE. Applicant: Bellwether Bio, Inc. Application EP 24183205.4, filed December 13, 2017. The sequence listing filed with the application follows.

SEQUENCE LISTING (4 sequences)

SEQ ID NO: 1 - DNA, 17 bp, synthetic construct
  misc_feature 1..17: note = Synthetic: Adapter 2.1
  modified_base 17: mod_base = OTHER; note = Dideoxythymidine [ddT]
  source 1..17: mol_type = other DNA
cgacgctcttccgatct

SEQ ID NO: 2 - DNA, 34 bp, synthetic construct
  misc_feature 1..34: note = Synthetic: Adapter 2.2
  modified_base 1: mod_base = OTHER; note = 5Phos
  modified_base 30..34: mod_base = OTHER; note = Phosphorothioate bond
  source 1..34: mol_type = other DNA
agatcggaagagcgtcgtgtagggaaagagtgta

SEQ ID NO: 3 - DNA, 10 bp, synthetic construct
  misc_feature 1..10: note = Synthetic: biotin-conjugated adapter oligo CL78
  modified_base 1: mod_base = OTHER; note = 5Phos
  modified_base 10: mod_base = OTHER; note = 10 - Int C3 Spacers, 3BioTEG
  source 1..10: mol_type = other DNA
agatcggaag

SEQ ID NO: 4 - DNA, 34 bp, synthetic construct
  misc_feature 1..34: note = Synthetic: oligo CL9
  source 1..34: mol_type = other DNA
gtgactggagttcagacgtgtgctcttccgatct